European Patent Specification EP 3 866 606 B1, published May 1, 2024. Title: LACTASE ENZYMES WITH IMPROVED PROPERTIES AT ACIDIC PH. Applicant: Chr. Hansen A/S. The sequence listing filed with the application follows.

SEQUENCE LISTING (28 sequences)

SEQ ID NO: 1 - protein, 698 aa, Bifidobacterium adolescentis
MRRNFEWPKLLTADGRGIAFGGDYNPDQWSEDIWDDDIRLMKQAGVNTVALAIFSWDRIQPTEDRWDFGWLDRIIDKLGNAGIAVDLASATATAPLWLYESHPEVLPRDKYGHPVNAGSRQSWSPTSPVFKEYALTLCRKLAERYGTNPYVTAWHMGNEYGWNNREDYSDNALDAFRAWCRRKYGTIGALNQAWGTTFWGQEMNGFDEVLIPRFMGADSMVNPGQKLDFERFGNDMLLDFYKAERDAIAEICPDKPFTTNFMVSTDQCCMDYAAWAEEVNFVSNDHYFHEGESHLDELACSDALMDSLALGKPWYVMEHSTSAVQWKPLNTRKRKGETVRDSLAHVAMGADAINFFQWRASAFGAESFHSAMVPHAGEDTKLFRQVCELGASLHTLADAGVQGTELAHSDTAILFSAESEWATRSQTLPSMKLNHWHDVRDWYRAFLNAGSRADIVPLAYDWSSYKTVVLPTVLILSAADTQRLADFAAAGGRVVVGYATGLIDEHFHTWLGGYPGAGDGLLRSMLGVRGEEFNILGAEAEGEPGEIRLSSADDSAALDGTTTRLWQNDVNVTGEHAQVLATYAGEEADEWELDGTAAVTRNPYGSGEAYFVGCDLDVADLTKLVRAYLAAPSQDNADVLHTVRESADATFDFYLPRGKETVELQGIEGEPVILFQTERGKKPGSYTVHRNGVLVVRR

SEQ ID NO: 2 - protein, 690 aa, Bifidobacterium adolescentis
MNQRREHRWPRPLEGRRARIWYGGDYNPDQWPEEVWDEDVRLMVKAGVNLVSVGIFSWAKIEPREDMYDFGWLDRIIDKLGKAGIAVDLASATASPPMWLTQAHPEVLWKDYRGDVCQPGARQHWRPTSPVFCEYALKLCRAMAEHYKDNPYVVAWHVGNEYGCHNRFDYSEDAERAFQDWCEERYGTIEAVNDAWGTAFWAQHLNDFSEIVPPRFIGDGNFMNPGKLLDFKRFSSDALKSFYVAERDALAEITPEKPLTTNFMVSAGGSVLDYDDWGGEVDFVSNDHYFIPGEAHLDELAFSASLVDGISRKDPWFLMEHSTSAVNWRPINYRKEPGQLVRDSLAHVAMGADAVCYFQWRQSRSGAEKFHSAMLPHAGEDSQTFRDVCELGRDLGTLADEGLLGTKLAKSSVAIVFDYESEWASEHTATPTQNVHHIDEPLAWFRALADVGVTADVVPIRSNWDEYDVAILPSVYILSEENTRRVRDYVANGGKLIATYYTGISDERDHVWLGGYPGSIRDVVGVRIEEFAPMGSDWPGVPDHLDLDNGAVAHDIVDVIGSIGKDAKVLASFKDDPWTGMDGRPAIVSNPYGEGRSVYVGARLGRDGIARSLPMILETLGVEVKDSSDPDLLRIERVDESTGARFTFLFNRTKEPVSMLVEGRPVVMSLADCAGATVTINPNGVLVVKQ

SEQ ID NO: 3 - protein, 698 aa, Bifidobacterium adolescentis
MRRNFEWPKLLTADGRGIAFGGDYNPDQWSEDIWDDDIRLMKQAGVNTVALAIFSWDRIQPTEDRWDFGWLDRIIDKLGNAGIAVDLASATATAPLWLYESHPEVLPRDKYGHPVNAGSRQSWSPTSPVFKEYALTLCRKLAERYGTNPYVTAWHMGNEYGWNNREDYSDNALDAFRAWCRRKYGTIGALNQAWGTTFWGQEMNGFDEVLIPRFMGADSMVNPGQKLDFERFGNDMLLDFYKAERDAIAEICPDKPFTTNFMVSTDQCCMDYAAWAEEVNFVSNDHYFHEGKSHLNKLACSDALMDSLALGKPWYVMEHSTSAVQWKPLNTRKRKGETVRDSLAHVAMGADAINFFQWRASAFGAESFHSAMVPHAGEDTKLFRQVCELGASLHTLADAGVQGTELAHSDTAILFSAESEQATRSQTLPSMKLNHWHDVRDWYRAFLDAGSRADIVPLAYDWSSYKTVVLPTVLILSAADTQRLADFAAAGGRVVIGYATGLIDEHFHTWLGGYPGAGDGLLRLMLGVRGEEFNILGAEAEGEPSEIRLASADDSVAMDGSTTRLWQNDVNVTGEHAQVLATYAGEEADEWELDGTAAVTRNPYGSGEAYFVGCDLDVADLTKLVRAYLAAPSQDNADVLHTVRESADATFDFYLPRGKETVELQGIEGEPVILFQTERGKKPGSYTVHRNGVLVVRR

SEQ ID NO: 4 - protein, 668 aa, Lactobacillus amylovorus
MTKTLSRFLYGGDYNPDQWTEETWPEDIKVFKKVDLNSATINIFSWAVLEPREGVYDFSKLDKIVQELSDANFDIVMGTATAAMPAWMFKKYPDIARVDYQGRRHVFGQRHNFCPNSKNYQRLDSELVEKLAQHYADNSHIVVWHVNNEYGGNCYCGNCQNAFRDWLRNKYKTLGALNKAWNMNVWSHTIYDWDEIVVPNELGDAWGPESSETIVAGLSIDYLRFQSESLQNLFKMEKAVIKKYDPETPVTTNFHSLPNKMIDYQKWAKDQDIISYDSYPTYDAPAYKPAFLYDLMRSLKHQPFMLMESAPSQVNWQSYSPLKRPGQMAATELQAVAHGADTVQFFQLKQAVGGSEKFHSAIIAHSQRTDTRAFCELADLGQKLKEAGPTILGSKTKAKVAIVFDWSNFWSYEYVDGITQDLNYVDSILDYYRQFYERNIPTDIIGVDDDFSNYDLVVAPVLYMVKAGLAEKINSYVEKGGHLVTTYMSGMVDSTDNVYLGGYPGPLKDVTGIWVEESDAMVPGQKVRVTMDGKEYETNLMCDLIHPNKAKVLASYADEFYTGTAAITENDYGKGKAWYVGTKLGHQGLTQLFNHIVLETGVESLVCDSHKLEVTKRVTADGKELYFVLNMSNEERELPNKFADYEDILTGEKAKSSMKGWDVQVLTK

SEQ ID NO: 5 - protein, 626 aa, Lactobacillus amylovorus
MKANIKWLDDPEVFRINQLPAHSDHPFYKDYREWQNHSSSFKQSLNGAWQFHFSKDPQSRPIDFYKRSFDSSSFDTIPVPSEIELNGYAQNQYTNILYPWESKIYRKPAYTLGRGIKDGDFSQGKDNTVGSYLKHFDLNPALAGHDIHIQFEGVERAMYVYLNGHFIGYAEDSFTPSEFDLTPYIQAKDNILAVEVFKHSTASWLEDQDMFRFSGIFRSVELLALPRTHLMDLDIKPTVVNDYHDGVFNAKLHFMGKTSGNVHVLIEDIDGKTLLNKKLPLKSTVEIENETFANVHLWDNHDPYLYQLIIEVHDQDGKLVELIPYQFGFRKIEITKDHVVLLNGKRLIINGVNRHEWDAKRGRSITLADMKQDIATFKHNNINAVRTCHYPNQIPWYYLCDQNGIYMMAENNLESHGTWQKLGQVEATSNVPGSIPEWREVVVDRARSNYETFKNHTAILFWSLGNESYAGSNIAAMNKLYKDHDSSRLTHYEGVFHAPEFKKEISDLESCMYLPPKEAEEYLQNPKKPLVECEYMHDMGTPDGGMGSYIKLIDKYPQYMGGFIWDFIDQALLVHDPVSGQDVLRYGGDFDDRHSDYEFSGDGLMFADRTPKPAMQEVRYYYGLHK

SEQ ID NO: 6 - protein, 316 aa, Lactobacillus amylovorus
MAYTNNLHVVYGEASLGVNGQDFAYLFSYERGGLESLKIKDKEWLYRTPTPTFWRATTDNDRGSGFNQKAAQWLGADMFTKCVGIHVQVDDHRFDELPVAPINNQFSNQEFAHEVKVAFDYETLTTPATKVKIIYNINDFGHMTITMHYFGKKGLPPLPVIGMRFIMPTKAKSFDYTGLSGETYPDRMAGAERGTFHIDGLPVTKYLVPQENGMHMQTNELVITRNSTQNNADKDGDFSLKITQTKQPFNFSLLPYTAEELENATHIEELPLARRSVLVIAGAVRGVGGIDSWGSDVEEQYHIDPEQDHEFSFTLN

SEQ ID NO: 7 - protein, 693 aa, Bifidobacterium bifidum
MERNMSKRRKHSWPQPLKGAESRLWYGGDYNPDQWPEEVWDDDIRLMKKAGVNLVSVGIFSWAKIEPEEGKYDFDWLDRAIDKLGKAGIAVDLASATASPPMWLTQAHPEVLWKDERGDTVWPGAREHWRPTSPVFREYALNLCRRMAEHYKGNPYVVAWHVSNEYGCHNRFDYSDDAMRAFQKWCKKRYKTIDAVNEAWGTAFWAQHMNDFSEIIPPRYIGDGNFMNPGKLLDYKRFSSDALKELYIAERDVLESITPGLPLTTNFMVSAGGSMLDYDDWGAEVDFVSNDHYFTPGEAHFDEVAYAASLMDGISRKEPWFQMEHSTSAVNWRPINYRAEPGSVVRDSLAQVAMGADAICYFQWRQSKAGAEKWHSSMVPHAGEDSQIFRDVCELGADLGRLSDEGLMGTKTVKSKVAVVFDYESQWATEYTANPTQQVDHWTEPLDWFRALADNGITADVVPVRSDWDSYEIAVLPCVYLLSEETSRRVREFVANGGKLFVTYYTGLSDENDHIWLGGYPGSIRDVVGVRVEEFAPMGNDMPGALDHLDLDNGTVAHDFADVITSTADTSTVLASYKAERWTGMNEVPAIVANGYGDGRTVYVGCRLGRQGLAKSLPAMLGSMGLSDLAGDGRVLRVERADAAAASHFEFVFNRTHEPVTVDVEGEAIAASLAHVDDGRATIDPTGVVVLRR

SEQ ID NO: 8 - protein, 680 aa, Lactobacillus brevis
MKRELKSKVFLHGGDYNPEQWLGEPEIINEDFALFKNAAINTVTVGIFSWAKLEPEEGKYDFAWLDDIFDRVEKMNGYVILATPSGARPAWLARKYPEVLRTDFNNQKRGFGGRHNHCLTSPIYRKKVREINTKLAEHFGKRPSLILWHISNEYSGECYCDLCQQAFRDWLKKKYRTLERLNHSWWNTFWSHTFSDWNQIHAPSPLSEMGNKGMNLDWKRFVSDQAISFIDNEVEPLRKITSEIPVTTNMMAGNPLMDPFTGYNYQEMAKHLDVISWDSYPLWGNDFQSTEKLGQNVGLIHDFFRSLKHQNFMIMENTPSRVNWADIDRAKRPGMHQLASLQDIAHSSDSVLYFQLRASRGSAEMFHGAVIEHRHPEKTRVFHDVKDVGHDLEKLESIYSTSYTKAKVGIVYDYNNIWALEDAEGYSKDKKIWQTIQSQYQYFYQNDIPVDFVSPNDNFTQYKLLIDPMHFLMTKEYMDKLESFVKKCGYVVGTYISGVVDENGLAYMNEWPKQLQSIYGIEPLETDSLYPKQSNSIEFAGHRYQAYDFCETIFKHDAKVLAKYTTDFYSGTPALTAHKCGEGKGYYIACRTDTDFLSAIYGQIVKELDLLPNLPIKKETTKISLQVRENDDEKYLFVQNFSHEQQSILLKQKMKEMLSDEFEENKVIVKPYGTKIYQMN

SEQ ID NO: 9 - protein, 689 aa, Bifidobacterium catenulatum
MTQRRSYRWPQPLAGQQARIWYGGDYNPDQWPEEVWDDDVRLMKKAGVNLVSVGIFSWAKIETSEGVYDFDWLDRIIDKLGEAGIAVDLASATASPPMWLTQAHPEVLWKDYRGDVCQPGARQHWRPTSPVFREYALKLCRAMAEHYKGNPYVVAWHVSNEYGCHNRFDYSEDAERAFRKWCEERYGTIDAVNDAWGTAFWAQRMNDFTEIVPPRFIGDGNFMNPGKLLDFKRFSSDALKAFYVAERDALAEITPDLPLTTNFMVSAAGSVLDYDDWGREVDFVSNDHYFIPGEAHLDELAFSASLVDGIARKDPWFLMEHSTSAVNWRPVNYRKEPGQLVRDSLAHVAMGADAVCYFQWRQSKAGAEKFHSAMVPHTGEDSAVFRDVCELGADLNTLADNGLLGTKLAKSKVAVVFDYESEWATEHTATPTQKVHHVDEPLQWFRALADHGVTADVVPVSSNWDEYEVVVLPSVYILSEETTRRVRDYVVNGGRLIVTYYTGLSDEKDHVWLGGYPGSIRDVVGVRVEEFMPMGDDFPGVPDCLGLSNGAVAHDIADVIGSVDGTATVLETFRDDPWTGMDGAPAIVANTFGEGRSVYVGARLGRDGIAKSLPEIFESLGMAETGENDSRVLRVEREGSDGSRFVFSFNRTHEAVQIPFEGKIVVSSFAEVSGENVSIKPNGVIVTKQ

SEQ ID NO: 10 - protein, 689 aa, Bifidobacterium pseudocatenulatum
MTQRRAYRWPQPLAGQQARIWYGGDYNPDQWPEEVWDDDVRLMKKAGVNLVSVGIFSWAKIETSEGVYDFDWLDRIINKLGEAGIAVDLASATASPPMWLTQAHPEVLWKDYRGDVCQPGARQHWRPTSPVFREYALKLCRAMAEHYKGNPYVVAWHVSNEYGCHNRFDYSEDAERAFRKWCEERYGTIDAVNDAWGTAFWAQRMNDFTEIVPPRFIGDGNFMNPGKLLDFKRFSSDALKAFYVAERDALAEITPDLPLTTNFMVSAAGSVLDYDDWGREVDFVSNDHYFIPGEAHLDELAFSASLVDGIARKDPWFLMEHSTSAVNWRPVNYRKEPGQLVRDSLAHVAMGADAVCYFQWRQSKAGAEKFHSAMVPHAGEDSAVFRDVCELGADLNTLADNGLLGTKLAKSKVAVVFDYESEWASEHTATPTQKVHHVDEPLQWFRALADHGVTADVVPVRGAWDDYEMVVLPSVYLLSEETTRRVRDYVVGGGRLVVTYYTGISDEKDHVWLGGYPGSIRDVVGVRVEEFMPMGDDFPGVPDCLGLSNGAVAHDIADVIGSVDGTATVLETFKDDPWTGMDGAPAIVAHTFGEGRSVYVGARLGRDGIALSLPEILDSLGMAEAGGNDGRVLRVEREGADGSRFVFSFNRTHETVRVPVEGEVVVSSFAEVSGETISIKPNGVIVTKQ

SEQ ID NO: 11 - protein, 680 aa, Lactobacillus gasseri
MKRILNTNEFLHGGDYNPEQWWDEPDVINQDFALFKQAKINTVTVGIFSWAKLEPEEGNYDFSWLDSIFDRVEEMNGHVVLATPSGARPAWLAQKYPEVLRTDNLGNKRGFGGRHNHCLTSPIYREKVREINTKLAEHFGQRKSLVLWHISNEYSGECYCESCKNAFRDWLKNKYGNLDNLNHAWWNTFWSHTYNDWSQVNPPSPLGEMGNKGMNLDWKRFITDQTISFIDNEAAPLRKITPNVPVTTNMMAGNPLMDPFAGFDYQKVAKHLDFISWDSYPAWGNDNQTTAELGRNVGLVHDFFRSLKHQNFLVMENTPSRVNWHSVDRAKRPGMHELASLQDVARGSQGVLYFQLRASRGSSEMFHGAVIEHLHPEQTRAFKDVTTVGKDLENIRPIINTNYAKARVAIVFSYDSYWALQDAESYSKDKKIWQTIQKHYRYFYKHDIPVDFVSVEDDFSNYDLLIDPMHFLMSKAYLKKLASYVKNGGRVVGTYISGVVDENDLAYMNEWPKELQDIYGVEPLETDVLYPGQSNTLNFDGHEYKAHDYCETLINCRGKVLAKYASDFYQDTPAVVEHEYGAGKGYYLACRTDYDLLEKFYEKITANLIPEFPVKKFSSNISIQVRENKDQKYYFVQNFSDKSEQIKVDGELEDLLEKKIDRGEVVLNPFGSKIYYKKGN

SEQ ID NO: 12 - protein, 621 aa, Lactobacillus helveticus
MLEPEEGKYDFSELDKVVKKLSDANFDIVIGTSTAAMPAWMFKKYPDVARVDYQGRRHVFGQRYNFCPNSKNYQRLAGNLVEELAKHYQNNPNIVVWHVNNEYGGNCYCENCQHEFRKWLKDKYQTLDALNKAWNMNVWSHTIYDWDEIVVSNELGDAWGPEGSETIVAGLSIDYLRFQSESLQNLFKMEKQIIKKHDSEAPVTTNFHSLPNKMIDYQKWAKDQDIISYDSYHTYDAPTYKPAFLYNLMRSLKHQPFMLMESAPSQVNWQPYSPLKRPGQMAATELQAVAHGADTVQFFQLKQAVGGSEKFHSAVIAHSQRTDTRVFKELVDLGHKLKRAGSTILGSTINAKVGIVFDWSNFWSYEYVDGISQDMDYVDSILDYYRQFYERNIPTDIISVDDDFSKYDLIVAPVLYMVKDGLAEKINNYVECGGNFVTTYMSGMVDSTDNVYLGGYPGPLKNVTGIWVEESDAVVPGHTTTVSLKGKDYKAGFVCDLIHPEQAKVLAEYSNEFYAGTPAITENKYGQGKAWYVGTRLDHTGLTQLFNHIVLESNIESLVCDGDKLEVTKRVTQDGQELYFVLNMSNEVRNLPQKFIGYQDILTDKKASDKLERWGVQVLTK

SEQ ID NO: 13 - protein, 710 aa, Bifidobacterium longum
MTTHRAFRWPSLLTESGRGIAFGGDYNPDQWPEETLDEDIRLMGEAGVNVVSLAIFSWDKIEPVEGAFTFEWLDHVIDRLGRAGIAVDLASATAAAPLWLYESHPEVLPVDRYGHTVNAGSRQSWQPTSPVFKEYALRLCRKLAEHYKDNPYVTAWHMGNEYGWNNRYDYSDNALAAFRTWCEAKYGTIDALNEAWGTAFWSQHVNSFDEVLLPRHMGGDAMVNPSQQLDYERFGNDMLLDFYKAERDAIEQICPDKPFTTNFMVSTDQCVMNYAKWADEVDFVSNDHYFHEGESHLDELACSDALMDSLALGKPWYVMEHSTSAVQWKPLNTRKRAGELMRDSLAHVAMGADAICFFQWRQSKSGAEAFHSAMLPHAGADSKVFRGVCELGKALKTLSDAGLQGTELERAGTAILFSAESEWATRSETLPSMKLNHWHDVRDWYRGFLDAGLRADVVPLAYDWTGYKTIVLPTVLSLSDEDVLRIADFAKAGGTVIVGYAAGLIDEHFHIGLGGYPGAGNGLLRDMLGIRSEEFNILGEEAEGEPSEISLSNGLTTRLWQNDVTSVAADTTVLASYAGESAADWELERTPAITSRPYGNGTAIYVGCDLNRHDIAQLLKALGSRWQELSAQPTESGQTPTYPTTDPRILHTIRRSADGSTRFDFYLNRSNQPVAINGVEGDPIIAHRCETDAVGYTLNRNAILIAKTSC

SEQ ID NO: 14 - protein, 691 aa, Bifidobacterium longum
MERKEFKWPQPLAGNKPRIWYGGDYNPDQWPEEVWDEDVALMQQAGVNLVSVAIFSWAKLEPEEGVYDFDWLDRVIDKLGKAGIAVDLASGTASPPMWMTQAHPEILWVDYRGDVCQPGARQHWRATSPVFLDYALSLCRKMAEHYKDNPYVVSWHVSNEYGCHNRFDYSEDAERAFQKWCEKKYGTIDAVNDAWGTAFWAQRMNNFSEIIPPRFIGDGNFMNPGKLLDWKRFSSDALLDFYKAERDALLEIAPKPQTTNFMVSAGGTGIDYDKWGYDVDFVSNDHYFTPGEAHFDELAYSASLCDGIARKNPWFLMEHSSSAVNWRPINYRVEPGELVRDSLAHLAMGSDAICYFQWRQSKAGAEKWHSSMVPHAGPDSQIFRDVCELGADLNKLADEGLLSTKLVKSKVAVVFDYESQWVTEHTATPTQEVRHWTEPLAWFRALADNGLTADVVPVRGSWDEYEAVVLPSLTILSEETTRRVREYVANGGKLFVTYYTGLVDDKDHVWLGGYPGSIRDVVGVRVEEFAPMGNDFPGAMDHLDLDNGTVAHDFADVITSVADTAHVVASFKADKWTGFDGAPAITVNDFGDGKAAYVGARLGREGLAKSLPALLEELGIETSAEDDRGEVLRVERADETGENHFVFLFNRTHDVAVVDVEGEPLVASLAQVNESERTAAIQPNGVLVVKL

SEQ ID NO: 15 - protein, 719 aa, Bifidobacterium longum
MTTRRTFRWPSLLTESGRGIAFGGDYNPDQWPEETLDEDIRLMVQAGVNTVALAIFSWDKIEPREGEFTFEWLDHVIDKLGAASIAVDLASATATAPLWLYERHPEVLPIDRYGHVVNAGSRQSWQPTSPVLKEYALRLCRKLAEHYKDNPYVTAWHMGNEYGWNNRYDYSDNALAAFRTWCEAKYGTVDALNEAWGTAFWSQHVNSFDEVLLPRHMGGDSMVNPPQQLDYERFGNDMLLDFYKAERDAIEEICPGKPFTTNFMVSTDQCTMDYAQWANEVDFVSNDHYFHEGESHLDELACSDALMDSLALGKPWYVMEHSTSAVQWKPLNTRKRAGELMRDSLAHVAMGADAINFFQWRQSASGAEAFHSAMVPHAGSDTKLFRGVCELGAALKTLSDAGVQDTELKRADTAILFSAESEWATRSETLPSMKLNHWHDVRDWYRGYLDAGARADVVPLAYDWSGYQTIVLPTVIALSDEDTRRIADFAENGGTVIVGYATGLIDEHFHIGLGGYPGAGNGLLRDMLGIRSEEFNILGEEAEDEPAEIGLSNGLTTRLWQNDVTSVAPDTRVLATYVGTAAADWELDGVPAITSHPHGQGAAIYVGCDLGRHDITHLLKELNTTAPSDERAPDQRPGGGEINAATTTAAATTHDPRILHTIRQSSDGTIRFDFYLNRSKQPVAVNGVEGDPIIAHRCETDAVGYTLNRNAILIAKTSC

SEQ ID NO: 16 - protein, 672 aa, Lactobacillus reuteri
MMKKELPRFLYGGDYNPEQWPEETWDEDIKVFKQADINSATINVFSWALLEPQEGKYDFTKLDKIIKELTVADFDIVLATSTAAMPAWMFKKYPDVARVDYQGRRHVFGARHNFCPSSKNYRRLAKNLVEQLAKRYGDNPHIVAWHVNNEYGGNCYCEECQTEFQQWLKARYQTLDNLNHAWNMNVWSHTIHDWNEIVVPNELGDAWGPEGSETIVAGLSIDYLRFQSAQMLDLFKMEKQIIEKYDPTTLVTTNFHSLPNKMIDYQQWASAQDIISYDSYPAYDAPIYQPAFLYDLMRSLKHQPFMLMESTPSQVNWQPYSPLKRPGQMAATELQAVAHGADTVQFFQLKQALGGSEKFHGAVISHANRTDTRVFKEVAKLGHDLRKVGPVIKDSQTKARVALIFDWSNFWSFEYVDGITQDLKYVPIILDYYRQFYELNIPTDVISVDDDFRQYDLVVAPVLYMVKGGLGKKITDYVANGGNFITSFMSGMVNESDNIYPGGYPGPLKDVMGLWVEESDAILPNKDVKLTMTTGDELTGYLIADLIRLNGAHVLAEYASEFYAGTPAVTENTYSKGKAWYVGSRLDHASLRKIIMHIVDDVHLSALVKEPTELEITKRQNSAGQDIYFVLNMGKGKQPLPVEFQKGYRDLLTGDSPETMLDSWDVEILVQE

SEQ ID NO: 17 - protein, 1007 aa, Lactobacillus delbrueckii subsp. lactis
MSNKLVKEKRVDQADLAWLTDPEVYEVNTIPPHSDHESFQSQEELEEGKSSLVQSLDGNWLIDYAENGQGPINFYAEDFDDSNFKSVKVPGNLELQGFGQPQYVNIQYPWDGSEEIFPPQVPSKNPLASYVRYFDLDEALWDKEVSLKFAGAATAIYVWLNGHFVGYGEDSFTPSEFMVTKFLKKEGNRLAVALYKYSSASWLEDQDFWRLSGLFRSVTLEAKPLLHLEDLKLTASLTDNYQKGKLEVEANIAYRLPNASFKLEVRDSEGDLVAEKVGPIRSEKLGFSLADLPVAAWSAEKPNLYQVRLYLYQAGSLLEVSRQEVGFRNFELKDGIMYLNGQRIVFKGVNRHEFDSKLGRAITEADMIWDIKTMKQSNINAVRCSHYPNQSLFYRLCDKYGLYVIDEANLESHGTWEKVGHEDPSFNVPGDDQHWLGASLSRVKNMMARDKNHASILIWSLGNESYAGTVFAQMADYVRKADPTRVQHYEGVTHNRKFDDATQIESRMYAPAKEIEEYLTKKPAKPFISVEYAHAMGNSVGDLAAYTALEKYPHYQGGFIWDWIDQGLEKDGHLLYGGDFDDRPTDYEFCGDGLVFADRTTSPKLANVKALYSNLKLEVKDGQLFIKNDNLFTNSSAYYFLASLLVDGKLTYQSQPLTFGLEPGESGTFVLPWPEVEDEKGEIVYQVTAHLKEDLPWADEGFTVAEAEEAVTKLPEFYPAGRPELVDSDFNLGLKGNGFRILFSKAKGWPVSIKYAGREYLKRLPEFTFWRALTDNDRGAGYGYDLAKWENAGKYARLQDISYEIKENSALVKTTFTLPVALKGDLTITYEVDSLGKIAVTANFPGAVENGLLPAFGLNFALPKELSDYRYYGLGPNESYADRLEGSYLGIYQGAVEKNFTPYLRPQEAGNRSKVRYYQLFDEEGGLEFTANGADLNLSALPYSAAQIEAADHAFELTNNYTWVRALAAQMGVGGDDSWGQKVHPEFCLDAQEARQLKLVIQPLLLK

SEQ ID NO: 18 - protein, 705 aa, Bifidobacterium angulatum
MAHRRTFHWPSLLTESGRGIAFGGDYNPDQWPEDVWDDDIRLMKQAGVNTVALAIFSWDRIQPEKHRWEFGWLDCIIDKLGKAGIAVDLASATATAPLWLYEQHPEVLPHDKYGHPINAGSRQSWSPTSPVFKEYALTLCRKLAERYGTNPYVTAWHMGNEYGWNNRYDYCDNALHAFRAWCERKYGTIEALNAAWGTTFWGQEMNGFDEVLIPRFMGADSMVNPGQKLDFERFGNDMLLDFYRAERDAIAEICPDKPFTTNFMVSTDQCCMDYADWANEVDFVSNDHYFHEGESHIDELFCSDALMDSLALGRPWYVMEHSTSAVQWKDLNIRKRKGETVRDSVAHVAMGADAINFFQWRASAFGAESFHSAMVPHAGEHTKLYRSVCELGAALKTLGDAGVQGSELVRSDTAILFSAESEWATRSETLPSKKLNHWHDVRDWYRAYLDAGTRADIVPLKYDWSGYATVVLPTVLMLSAADTARLERFVRDGGTVVVGYASGLIDENFHTWLGGYPGAGDGMLRTMLGIRGEEFNILGAQAEGEPSEIRLSNGMVTRLWQNDIAVDGADTEVLASYAGTQADEWELDGTAAITRNPYGKGMAYFVGCDLNVADLAVFVGDHLTVGQACEAGDGADYDPTITLHTERASAEAIFDFYLPRGKNETVVSGISGEPVYRFQCDEGEAPGVYTIRRNGVLVVKRYNRQ

SEQ ID NO: 19 - protein, 626 aa, Lactobacillus fermentum
MEAELKWLDDPEVFRVNQLPAHSDHRFYRDQEEAALEKSSYVQNLNGRWGFKFSKNPMERPVDFYKLDFDRNDFGEIEVPSEIELSNFAQINYTNITMPWTGKIYRRPAYTLGDNKEEGSFSQGQDNTVGSYVRHFTLAEGLKNHDVHVVFEGVERAMYVWLNGHFIGYAEDSFTPSEFDLTPYLVDGDNLLAVEVYKHATSSWIEDQDMFRFSGIFRDVNLVAQPSIHVQDLKINARVADDMKTGSLGLVLKMVGQPGSVQVEVADQTGAAVLNRQLNADGNWTMAPVQLVGIHLWDNHHPYLYQLTLTVRDATGRVVEVIPYQFGFRRVEIDQDKVLRLNGKRLIINGVNRHEWNCHRGRAVTIEDMHTDLGIFKENNINAVRTSHYPDQIPWYYLCDREGIYMMAENNLESHATWQKFGQDEPSYNVPGSLPQWKEAVVDRARSNYEIFKNHTAILFWSVGNESYAGEDILAMNNYYKEVDDTRPVHYEGVVHTKEYRDQISDFESWMYLPPKEVEAYLKKNPDKPFIECEYMHSMGNSVGGMGSYIKLLDKYPQYCGGFIWDFVDQAIEVVDPVTGQKSMRYGGDFDDHHADNEFSGDGICFADRTPKPAMQEVKYYYGLHK

SEQ ID NO: 20 - protein, 320 aa, Lactobacillus fermentum
MDYTNKLHVVYDDNILGLDGKDFQYLFSYEQGGPESFKIKGKEWLYRSPRPTFWRATTDNDRGNGFNVSSVQWLAADYVLPCQDIALQVDGKDKKLPLAPKTNRYSNQEFAKKVKITFTYQTQTVPATTVQVSYTVKASGKIKVNVHYTGAQLPSLPVLGWRMIMPTPATSFDYEGLSGETYPDRMAGGIEGTYHVEGLPVTPYLVPQENGMHMANKWVQITRATTLNNADPDAAPFRLKFEAPKKGKLNFSCLPYTSAELENATHPEELPAAHRTVLVIAGEVRGVGGIDSWGADVEEKYHIDATVDHDFSFKIVPELN

SEQ ID NO: 21 - protein, 1025 aa, Kluyveromyces lactis
MSCLIPENLRNPKKVHENRLPTRAYYYDQDIFESLNGPWAFALFDAPLDAPDAKNLDWETAKKWSTISVPSHWELQEDWKYGKPIYTNVQYPIPIDIPNPPTVNPTGVYARTFELDSKSIESFEHRLRFEGVDNCYELYVNGQYVGFNKGSRNGAEFDIQKYVSEGENLVVVKVFKWSDSTYIEDQDQWWLSGIYRDVSLLKLPKKAHIEDVRVTTTFVDSQYQDAELSVKVDVQGSSYDHINFTLYEPEDGSKVYDASSLLNEENGNTTFSTKEFISFSTKKNEETAFKINVKAPEHWTAENPTLYKYQLDLIGSDGSVIQSIKHHVGFRQVELKDGNITVNGKDILFRGVNRHDHHPRFGRAVPLDFVVRDLILMKKFNINAVRNSHYPNHPKVYDLFDKLGFWVIDEADLETHGVQEPFNRHTNLEAEYPDTKNKLYDVNAHYLSDNPEYEVAYLDRASQLVLRDVNHPSIIIWSLGNEACYGRNHKAMYKLIKQLDPTRLVHYEGDLNALSADIFSFMYPTFEIMERWRKNHTDENGKFEKPLILCEYGHAMGNGPGSLKEYQELFYKEKFYQGGFIWEWANHGIEFEDVSTADGKLHKAYAYGGDFKEEVHDGVFIMDGLCNSEHNPTPGLVEYKKVIEPVHIKIAHGSVTITNKHDFITTDHLLFIDKDTGKTIDVPSLKPEESVTIPSDTTYVVAVLKDDAGVLKAGHEIAWGQAELPLKVPDFVTETAEKAAKINDGKRYVSVESSGLHFILDKLLGKIESLKVKGKEISSKFEGSSITFWRPPTNNDEPRDFKNWKKYNIDLMKQNIHGVSVEKGSNGSLAVVTVNSRISPVVFYYGFETVQKYTIFANKINLNTSMKLTGEYQPPDFPRVGYEFWLGDSYESFEWLGRGPGESYPDKKESQRFGLYDSKDVEEFVYDYPQENGNHTDTHFLNIKFEGAGKLSIFQKEKPFNFKISDEYGVDEAAHACDVKRYGRHYLRLDHAIHGVGSEACGPAVLDQYRLKAQDFNFEFDLAFE

SEQ ID NO: 22 - protein, 1305 aa, Bifidobacterium bifidum
MVEDATRSDSTTQMSSTPEVVYSSAVDSKQNRTSDFDANWKFMLSDSVQAQDPAFDDSAWQQVDLPHDYSITQKYSQSNEAESAYLPGGTGWYRKSFTIDRDLAGKRIAINFDGVYMNATVWFNGVKLGTHPYGYSPFSFDLTGNAKFGGENTIVVKVENRLPSSRWYSGSGIYRDVTLTVTDGVHVGNNGVAIKTPSLATQNGGNVTMNLTTKVANDTEAAANITLKQTVFPKGGKTDAAIGTVTTASKSIAAGASADVTSTITAASPKLWSIKNPNLYTVRTEVLNGDTVLDTYDTEYGFRWTGFDATSGFSLNGEKVKLKGVSMHHDQGSLGAVANRRAIERQVEILQKMGVNSIRTTHNPAAKALIDVCNEKGVLVVEEVFDMWNRSKNGNTEDYGKWFGQTIAGDNAVLGGDKDETWAKFDLTSTINRDRNAPSVIMWSLGNEMMEGISGSVSDFPATSAKLVAWTKAADSTRPMTYGDNKIKANWNESNTMGDNLTANGGVVGTNYSDGANYDKIRTTHPSWAIYGSETASAINSRGIYNRTTGGAQSSDKQLTSYDNSAVGWGAVASSAWYDVVQRDFVAGTYVWTGFDYLGEPTPWNGTGSGAVGSWPSPKNSYFGIVDTAGFPKDTYYFYQSQWNDDVHTLHILPAWNENVVAKGSGNKVPVVVYTDAAKVKLYFTPKGSTEKRLIGEKSFTKKTTAAGYTYQVYEGTDKDSTAHKNMYLTWNVPWAEGTISAEAYDENNRLIPEGSTEGNASVTTTGKAAKLKADADRKTITADGKDLSYIEVDVTDANGHIVPDAANRVTFDVKGAGKLVGVDNGSSPDHDSYQADNRKAFSGKVLAIVQSTKEAGEITVTAKADGLQSSTVKIATTAVPGTSTEKTVRSFYYSRNYYVKTGNKPILPSDVEVRYSDGTSDRQNVTWDAVSDDQIAKAGSFSVAGTVAGQKISVRVTMIDEIGALLNYSASTPVGTPAVLPGSRPAVLPDGTVTSANFAVHWTKPADTVYNTAGTVKVPGTATVFGKEFKVTATIRVQRSQVTIGSSVSGNALRLTQNIPADKQSDTLDAIKDGSTTVDANTGGGANPSAWTNWAYSKAGHNTAEITFEYATEQQLGQIVMYFFRDSNAVRFPDAGKTKIQISADGKNWTDLAATETIAAQESSDRVKPYTYDFAPVGATFVKVTVTNADTTTPSGVVCAGLTEIELKTATSKFVTNTSAALSSLTVNGTKVSDSVLAAGSYNTPAIIADVKAEGEGNASVTVLPAHDNVIRVITESEDHVTRKTFTINLGTEQEFPADSDERD

SEQ ID NO: 23 - DNA, 30 bp, synthetic
  "combined DNA/RNA molecule"
  combined DNA/RNA molecule
attaaccaugcgacgcaacttcgaatggcc

SEQ ID NO: 24 - DNA, 31 bp, synthetic
  "combined DNA/RNA molecule"
  combined DNA/RNA molecule
atcttctcuttaccgccttaccacgagcacg

SEQ ID NO: 25 - DNA, 33 bp, synthetic
  "combined DNA/RNA molecule"
  combined DNA/RNA molecule
agagaagautttcagcctgatacagattaaatc

SEQ ID NO: 26 - DNA, 33 bp, synthetic
  "combined DNA/RNA molecule"
  combined DNA/RNA molecule
atggttaautcctcctgttagcccaaaaaacgg

SEQ ID NO: 27 - DNA, 22 bp, synthetic
cggcgtcacactttgctatgcc

SEQ ID NO: 28 - DNA, 20 bp, synthetic
ccgcgctactgccgccaggc